European Patent Application EP 4 752 229 A2, published June 3, 2026. Title: USE OF MULLERIAN INHIBITING SUBSTANCE (MIS) PROTEINS FOR CONTRACEPTION AND OVARIAN RESERVE PRESERVATION. Applicant: THE GENERAL HOSPITAL CORPORATION. Application EP. The sequence listing filed with the application follows.

SEQUENCE LISTING (23 sequences)

SEQ ID NO: 1 - DNA, 1680 bp, synthetic construct
  misc_feature 1..1680: note = Description of Artificial Sequence: Synthetic polynucleotide
  source 1..1680: mol_type = other DNA
atgaagtgggtgagcttcatcagcctgctgttcctgttcagcagcgcttactcccgcggtgtgttccgccgcagagcagaggagccagctgtgggcaccagtggcctcatcttccgagaagacttggactggcctccaggcagcccacaagagcctctgtgcctggtggcactgggcggggacagcaatggcagcagctcccccctgcgggtggtgggggctctaagcgcctatgagcaggccttcctgggggccgtgcagagggcccgctggggcccccgagacctggccaccttcggggtctgcaacaccggtgacaggcaggctgccttgccctctctacggcggctgggggcctggctgcgggaccctggggggcagcgcctggtggtcctacacctggaggaagtgacctgggagccaacaccctcgctgaggttccaggagcccccgcctggaggagctggccccccagagctggcgctgctggtgctgtaccctgggcctggccctgaggtcactgtgacgagggctgggctgccgggtgcccagagcctctgcccctcccgagacacccgctacctggtgttagcggtggaccgccctgcgggggcctggcgcggctccgggctggccttgaccctgcagccccgcggagaggactcccggctgagtaccgcccggctgcaggcactgctgttcggcgacgaccaccgctgcttcacacggatgaccccggccctgctcctgctgccgcggtccgagcccgcgccgctgcctgcgcacggccagctggacaccgtgcccttcccgccgcccaggccatccgcggaactcgaggagtcgccacccagcgcagaccccttcctggagacgctcacgcgcctggtgcgggcgctgcgggtccccccggcccgggcctccgcgccgcgcctggccctggatccggacgcgctggccggcttcccgcagggcctagtcaacctgtcggaccccgcggcgctggagcgcctactcgacggcgaggagccgctgctgctgctgctgaggcccactgcggccaccaccggggatcctgcgcccctgcacgaccccacgtcggcgccgtgggccacggccctggcgcgccgcgtggctgctgaactgcaagcggcggctgccgagctgcgaagcctcccgggtctgcctccggccacagccccgctgctggcgcgcctgctcgcgctctgcccaggtggccccggcggcctcggcgatcccctgcgagcgctgctgctcctgaaggcgctgcagggcctgcgcgtggagtggcgcgggcgggatccgcgcgggccgggtcgggcacggcgcagcgcgggggccaccgccgccgacgggccgtgcgcgctgcgcgagctcagcgtagacctccgcgccgagcgctccgtactcatccccgagacctaccaggccaacaattgccagggcgtgtgcggctggcctcagtccgaccgcaacccgcgctacggcaaccacgtggtgctgctgctgaagatgcaggcccgtggggccgccctggcgcgcccaccctgctgcgtgcccaccgcctacgcgggcaagctgctcatcagcctgtcggaggagcgcatcagcgcgcaccacgtgcccaacatggtggccaccgagtgtggctgccggtga

SEQ ID NO: 2 - DNA, 1704 bp, synthetic construct
  misc_feature 1..1704: note = Description of Artificial Sequence: Synthetic polynucleotide
  source 1..1704: mol_type = other DNA
atgaagtgggtgagcttcatcagcctgctgttcctgttcagcagcgcttactcccgcggtgtgttccgccgcagagcagaggagccagctgtgggcaccagtggcctcatcttccgagaagacttggactggcctccaggcagcccacaagagcctctgtgcctggtggcactgggcggggacagcaatggcagcagctcccccctgcgggtggtgggggctctaagcgcctatgagcaggccttcctgggggccgtgcagagggcccgctggggcccccgagacctggccaccttcggggtctgcaacaccggtgacaggcaggctgccttgccctctctacggcggctgggggcctggctgcgggaccctggggggcagcgcctggtggtcctacacctggaggaagtgacctgggagccaacaccctcgctgaggttccaggagcccccgcctggaggagctggccccccagagctggcgctgctggtgctgtaccctgggcctggccctgaggtcactgtgacgagggctgggctgccgggtgcccagagcctctgcccctcccgagacacccgctacctggtgttagcggtggaccgccctgcgggggcctggcgcggctccgggctggccttgaccctgcagccccgcggagaggactcccggctgagtaccgcccggctgcaggcactgctgttcggcgacgaccaccgctgcttcacacggatgaccccggccctgctcctgctgccgcggtccgagcccgcgccgctgcctgcgcacggccagctggacaccgtgcccttcccgccgcccaggccatccgcggaactcgaggagtcgccacccagcgcagaccccttcctggagacgctcacgcgcctggtgcgggcgctgcgggtccccccggcccgggcctccgcgccgcgcctggccctggatccggacgcgctggccggcttcccgcagggcctagtcaacctgtcggaccccgcggcgctggagcgcctactcgacggcgaggagccgctgctgctgctgctgaggcccactgcggccaccaccggggatcctgcgcccctgcacgaccccacgtcggcgccgtgggccacggccctggcgcgccgcgtggctgctgaactgcaagcggcggctgccgagctgcgaagcctcccgggtctgcctccggccacagccccgctgctggcgcgcctgctcgcgctctgcccaggtggccccggcggcctcggcgatcccctgcgagcgctgctgctcctgaaggcgctgcagggcctgcgcgtggagtggcgcgggcgggatccgcgcgggccgggtcgggcacggcgcagcgactacaaggatgacgacgacaaggcgggggccaccgccgccgacgggccgtgcgcgctgcgcgagctcagcgtagacctccgcgccgagcgctccgtactcatccccgagacctaccaggccaacaattgccagggcgtgtgcggctggcctcagtccgaccgcaacccgcgctacggcaaccacgtggtgctgctgctgaagatgcaggcccgtggggccgccctggcgcgcccaccctgctgcgtgcccaccgcctacgcgggcaagctgctcatcagcctgtcggaggagcgcatcagcgcgcaccacgtgcccaacatggtggccaccgagtgtggctgccggtga

SEQ ID NO: 3 - protein, 560 aa, Homo sapiens
MRDLPLTSLALVLSALGALLGTEALRAEEPAVGTSGLIFREDLDWPPGSPQEPLCLVALGGDSNGSSSPLRVVGALSAYEQAFLGAVQRARWGPRDLATFGVCNTGDRQAALPSLRRLGAWLRDPGGQRLVVLHLEEVTWEPTPSLRFQEPPPGGAGPPELALLVLYPGPGPEVTVTRAGLPGAQSLCPSRDTRYLVLAVDRPAGAWRGSGLALTLQPRGEDSRLSTARLQALLFGDDHRCFTRMTPALLLLPRSEPAPLPAHGQLDTVPFPPPRPSAELEESPPSADPFLETLTRLVRALRVPPARASAPRLALDPDALAGFPQGLVNLSDPAALERLLDGEEPLLLLLRPTAATTGDPAPLHDPTSAPWATALARRVAAELQAAAAELRSLPGLPPATAPLLARLLALCPGGPGGLGDPLRALLLLKALQGLRVEWRGRDPRGPGRAQRSAGATAADGPCALRELSVDLRAERSVLIPETYQANNCQGVCGWPQSDRNPRYGNHVVLLLKMQVRGAALARPPCCVPTAYAGKLLISLSEERISAHHVPNMVATECGCR

SEQ ID NO: 4 - protein, 559 aa, synthetic construct
  REGION 1..559: note = Description of Artificial Sequence: Synthetic polypeptide
MKWVTFISLLFLFSSAYSRGVFRRRAEEPAVGTSGLIFREDLDWPPGSPQEPLCLVALGGDSNGSSSPLRVVGALSAYEQAFLGAVQRARWGPRDLATFGVCNTGDRQAALPSLRRLGAWLRDPGGQRLVVLHLEEVTWEPTPSLRFQEPPPGGAGPPELALLVLYPGPGPEVTVTRAGLPGAQSLCPSRDTRYLVLAVDRPAGAWRGSGLALTLQPRGEDSRLSTARLQALLFGDDHRCFTRMTPALLLLPRSEPAPLPAHGQLDTVPFPPPRPSAELEESPPSADPFLETLTRLVRALRVPPARASAPRLALDPDALAGFPQGLVNLSDPAALERLLDGEEPLLLLLRPTAATTGDPAPLHDPTSAPWATALARRVAAELQAAAAELRSLPGLPPATAPLLARLLALCPGGPGGLGDPLRALLLLKALQGLRVEWRGRDPRGPGRARRSAGATAADGPCALRELSVDLRAERSVLIPETYQANNCQGVCGWPQSDRNPRYGNHVVLLLKMQVRGAALARPPCCVPTAYAGKLLISLSEERISAHHVPNMVATECGCR

SEQ ID NO: 5 - protein, 567 aa, synthetic construct
  REGION 1..567: note = Description of Artificial Sequence: Synthetic polypeptide
MKWVTFISLLFLFSSAYSRGVFRRRAEEPAVGTSGLIFREDLDWPPGSPQEPLCLVALGGDSNGSSSPLRVVGALSAYEQAFLGAVQRARWGPRDLATFGVCNTGDRQAALPSLRRLGAWLRDPGGQRLVVLHLEEVTWEPTPSLRFQEPPPGGAGPPELALLVLYPGPGPEVTVTRAGLPGAQSLCPSRDTRYLVLAVDRPAGAWRGSGLALTLQPRGEDSRLSTARLQALLFGDDHRCFTRMTPALLLLPRSEPAPLPAHGQLDTVPFPPPRPSAELEESPPSADPFLETLTRLVRALRVPPARASAPRLALDPDALAGFPQGLVNLSDPAALERLLDGEEPLLLLLRPTAATTGDPAPLHDPTSAPWATALARRVAAELQAAAAELRSLPGLPPATAPLLARLLALCPGGPGGLGDPLRALLLLKALQGLRVEWRGRDPRGPGRARRSDYKDDDDKAGATAADGPCALRELSVDLRAERSVLIPETYQANNCQGVCGWPQSDRNPRYGNHVVLLLKMQVRGAALARPPCCVPTAYAGKLLISLSEERISAHHVPNMVATECGCR

SEQ ID NO: 6 - protein, 24 aa, Homo sapiens
MKWVTFISLLFLFSSAYSRGVFRR

SEQ ID NO: 7 - DNA, 78 bp, Homo sapiens
  source 1..78: mol_type = genomic DNA
atgaagtgggtgagcttcatcagcctgctgttcctgttcagcagcgcttactcccgcggtgtgttccgccgcagagca

SEQ ID NO: 8 - protein, 18 aa, Homo sapiens
MKWVTFISLLFLFSSAYS

SEQ ID NO: 9 - protein, 18 aa, Homo sapiens
MKWVTFISLLFLFSSAYS

SEQ ID NO: 10 - protein, 18 aa, Homo sapiens
MKWVSFISLLFLFSSAYS

SEQ ID NO: 11 - protein, 21 aa, Homo sapiens
MKVSVAALSCLMLVTALGSQA

SEQ ID NO: 12 - protein, 17 aa, unidentified
  REGION 1..17: note = Description of Unknown: Stanniocalcin signal sequence
MLQNSAVLLLLVISASA

SEQ ID NO: 13 - protein, 19 aa, unidentified
  REGION 1..19: note = Description of Unknown: Invertase signal sequence
MLLQAFLFLLAGFAAKISA

SEQ ID NO: 14 - protein, 24 aa, synthetic construct
  REGION 1..24: note = Description of Artificial Sequence: Synthetic peptide
MKWVSFISLLFLFSSAYSRSLEKR

SEQ ID NO: 15 - protein, 24 aa, synthetic construct
  REGION 1..24: note = Description of Artificial Sequence: Synthetic peptide
MKWVSFISLLFLFSSAYSRSLDKR

SEQ ID NO: 16 - protein, 21 aa, synthetic construct
  REGION 1..21: note = Description of Artificial Sequence: Synthetic peptide
MNIFYIFLFLLSFVQGSLDKR

SEQ ID NO: 17 - protein, 19 aa, unidentified
  REGION 1..19: note = Description of Unknown: Immunoglobulin Ig signal sequence
MGWSCIILFLVATATGVHS

SEQ ID NO: 18 - protein, 29 aa, unidentified
  REGION 1..29: note = Description of Unknown: Fibulin B precursor signal sequence
MERAAPSRRVPLPLLLLGGLALLAAGVDA

SEQ ID NO: 19 - protein, 22 aa, unidentified
  REGION 1..22: note = Description of Unknown: Clusterin precursor signal sequence
MMKTLLLFVGLLLTWESGQVLG

SEQ ID NO: 20 - protein, 21 aa, unidentified
  REGION 1..21: note = Description of Unknown: Insulin-like growth factor-binding protein 4 signal sequence
MLPLCLVAALLLAAGPGPSLG

SEQ ID NO: 21 - protein, 8 aa, synthetic construct
  REGION 1..8: note = Description of Artificial Sequence: Synthetic peptide
DYKDDDDK

SEQ ID NO: 22 - DNA, 24 bp, synthetic construct
  misc_feature 1..24: note = Description of Artificial Sequence: Synthetic oligonucleotide
  source 1..24: mol_type = other DNA
gactacaaggatgacgacgacaag

SEQ ID NO: 23 - protein, 252 aa, synthetic construct
  REGION 1..252: note = Description of Artificial Sequence: Synthetic polypeptide
LELVPRGSGDPIEGRGGGGGDPKSCDKPHTCPLCPAPELLGGPSVFLFPPKPKDTLMISRTPEVTCVVVDVSHEDPEVKFNWYVDGVEVHNAKTKPREEQYNSTYRVVSVLTVLHQDWLNGKEYKCKVSNKALPAPIEKTISKAKGQPREPQVYTLPPSRDELTKNQVSLTCLVKGFYPSDIAVEWESNGQPENNYKATPPVLDSDGSFFLYSKLTVDKSRWQQGNVFSCSVMHEALHNHYTQKSLSLSPGK